European Patent Application EP 4 685 152 A1, published January 28, 2026. Title: LAG-3-binding peptide and uses thereof. Applicant: KYUNGPOOK NATIONAL UNIVERSITY INDUSTRY-ACADEMIC COOPERATION FOUNDATION. The sequence listing filed with the application follows.

SEQUENCE LISTING (2 sequences)

SEQ ID NO: 1 - protein, 9 aa, synthetic construct
CIRNDPAVC

SEQ ID NO: 2 - protein, 9 aa, synthetic construct
CSVLNASGC